European Patent Application EP 4 379 043 A1, published June 5, 2024. Title: 혈액 적합성을 갖는 중간엽 줄기세포, 이의 제조방법 및 용도. Applicant: TOOLGEN INCORPORATED. Application KR. The sequence listing filed with the application follows.

SEQUENCE LISTING (53 sequences)

SEQ ID NO: 1 - DNA, 23 bp, Homo sapiens
  source 1..23: mol_type = genomic DNA
gccccgagaccgccgtcgctcgg

SEQ ID NO: 2 - DNA, 23 bp, Homo sapiens
  source 1..23: mol_type = genomic DNA
tccgagcgacggcggtctcgggg

SEQ ID NO: 3 - DNA, 23 bp, Homo sapiens
  source 1..23: mol_type = genomic DNA
gagcaggagcgtccgagcgacgg

SEQ ID NO: 4 - DNA, 23 bp, Homo sapiens
  source 1..23: mol_type = genomic DNA
ctcggacgctcctgctcggctgg

SEQ ID NO: 5 - DNA, 23 bp, Homo sapiens
  source 1..23: mol_type = genomic DNA
tgggtcttcgcccaggtggccgg

SEQ ID NO: 6 - DNA, 23 bp, Homo sapiens
  source 1..23: mol_type = genomic DNA
gcccaggtggccggcgcttcagg

SEQ ID NO: 7 - DNA, 23 bp, Homo sapiens
  source 1..23: mol_type = genomic DNA
gtccgagcgacggcggtctcggg

SEQ ID NO: 8 - DNA, 23 bp, Homo sapiens
  source 1..23: mol_type = genomic DNA
cgtccgagcgacggcggtctcgg

SEQ ID NO: 9 - DNA, 23 bp, Homo sapiens
  source 1..23: mol_type = genomic DNA
gtagacttgattgacgggtttgg

SEQ ID NO: 10 - DNA, 23 bp, Homo sapiens
  source 1..23: mol_type = genomic DNA
acagtgtagacttgattgacggg

SEQ ID NO: 11 - DNA, 23 bp, Homo sapiens
  source 1..23: mol_type = genomic DNA
cacatccttcacaatctcgtcgg

SEQ ID NO: 12 - DNA, 23 bp, Homo sapiens
  source 1..23: mol_type = genomic DNA
ggatgtgaagcagacgtacttgg

SEQ ID NO: 13 - DNA, 23 bp, Homo sapiens
  source 1..23: mol_type = genomic DNA
ggcacgggtcttctcctacccgg

SEQ ID NO: 14 - DNA, 23 bp, Homo sapiens
  source 1..23: mol_type = genomic DNA
cgggacccggggccaggcagggg

SEQ ID NO: 15 - DNA, 23 bp, Homo sapiens
  source 1..23: mol_type = genomic DNA
cgcgggacccggggccaggcagg

SEQ ID NO: 16 - DNA, 23 bp, Homo sapiens
  source 1..23: mol_type = genomic DNA
caggagcgtccgagcgacggcgg

SEQ ID NO: 17 - DNA, 23 bp, Homo sapiens
  source 1..23: mol_type = genomic DNA
gtcgctcggacgctcctgctcgg

SEQ ID NO: 18 - DNA, 23 bp, Homo sapiens
  source 1..23: mol_type = genomic DNA
tcggacgctcctgctcggctggg

SEQ ID NO: 19 - DNA, 23 bp, Homo sapiens
  source 1..23: mol_type = genomic DNA
tggcagcatataatttaacttgg

SEQ ID NO: 20 - DNA, 23 bp, Homo sapiens
  source 1..23: mol_type = genomic DNA
tagacttgattgacgggtttggg

SEQ ID NO: 21 - DNA, 23 bp, Homo sapiens
  source 1..23: mol_type = genomic DNA
cctcaccgacgagattgtgaagg

SEQ ID NO: 22 - DNA, 23 bp, Homo sapiens
  source 1..23: mol_type = genomic DNA
ccttcacaatctcgtcggtgagg

SEQ ID NO: 23 - DNA, 23 bp, Homo sapiens
  source 1..23: mol_type = genomic DNA
tgaagcagacgtacttggcacgg

SEQ ID NO: 24 - DNA, 23 bp, Homo sapiens
  source 1..23: mol_type = genomic DNA
gaagcagacgtacttggcacggg

SEQ ID NO: 25 - DNA, 23 bp, Homo sapiens
  source 1..23: mol_type = genomic DNA
cgggtcttctcctacccggcagg

SEQ ID NO: 26 - DNA, 23 bp, Homo sapiens
  source 1..23: mol_type = genomic DNA
ctcctacccggcagggaatgtgg

SEQ ID NO: 27 - DNA, 23 bp, Homo sapiens
  source 1..23: mol_type = genomic DNA
gtgctctccacattccctgccgg

SEQ ID NO: 28 - DNA, 23 bp, Homo sapiens
  source 1..23: mol_type = genomic DNA
gtggagagcaccggttctgctgg

SEQ ID NO: 29 - DNA, 23 bp, Homo sapiens
  source 1..23: mol_type = genomic DNA
tggagagcaccggttctgctggg

SEQ ID NO: 30 - DNA, 23 bp, Homo sapiens
  source 1..23: mol_type = genomic DNA
ggagagcaccggttctgctgggg

SEQ ID NO: 31 - DNA, 23 bp, Homo sapiens
  source 1..23: mol_type = genomic DNA
tctggggagttctcatacagagg

SEQ ID NO: 32 - DNA, 23 bp, Homo sapiens
  source 1..23: mol_type = genomic DNA
caggtaaggtgtgaactctgggg

SEQ ID NO: 33 - DNA, 23 bp, Homo sapiens
  source 1..23: mol_type = genomic DNA
ccaggtaaggtgtgaactctggg

SEQ ID NO: 34 - DNA, 23 bp, Homo sapiens
  source 1..23: mol_type = genomic DNA
tccaggtaaggtgtgaactctgg

SEQ ID NO: 35 - DNA, 23 bp, Homo sapiens
  source 1..23: mol_type = genomic DNA
aacaattcagagttttgaacagg

SEQ ID NO: 36 - DNA, 23 bp, Homo sapiens
  source 1..23: mol_type = genomic DNA
atgtgaccgtagaagatgaacgg

SEQ ID NO: 37 - DNA, 23 bp, Homo sapiens
  source 1..23: mol_type = genomic DNA
taaagtccgttcatcttctacgg

SEQ ID NO: 38 - DNA, 23 bp, Homo sapiens
  source 1..23: mol_type = genomic DNA
atgaacggactttagtcagaagg

SEQ ID NO: 39 - DNA, 23 bp, Homo sapiens
  source 1..23: mol_type = genomic DNA
acaacactttcctaagcctccgg

SEQ ID NO: 40 - DNA, 23 bp, Homo sapiens
  source 1..23: mol_type = genomic DNA
caacactttcctaagcctccggg

SEQ ID NO: 41 - DNA, 23 bp, Homo sapiens
  source 1..23: mol_type = genomic DNA
attctacatcattggagctgtgg

SEQ ID NO: 42 - DNA, 23 bp, Homo sapiens
  source 1..23: mol_type = genomic DNA
cattggagctgtggtatttgtgg

SEQ ID NO: 43 - DNA, 23 bp, Homo sapiens
  source 1..23: mol_type = genomic DNA
acttgtgtagagatatagccagg

SEQ ID NO: 44 - DNA, 20 bp, synthetic construct
  source 1..20: mol_type = other DNA
ttcagcccaacctccccagc

SEQ ID NO: 45 - DNA, 20 bp, synthetic construct
  source 1..20: mol_type = other DNA
cccgctgccagccaggactg

SEQ ID NO: 46 - DNA, 22 bp, synthetic construct
  source 1..22: mol_type = other DNA
atacatcaatacattcgagtgc

SEQ ID NO: 47 - DNA, 19 bp, synthetic construct
  source 1..19: mol_type = other DNA
cttgttcagcataggacag

SEQ ID NO: 48 - DNA, 20 bp, synthetic construct
  source 1..20: mol_type = other DNA
gcactaagtcaggagattgg

SEQ ID NO: 49 - DNA, 20 bp, synthetic construct
  source 1..20: mol_type = other DNA
gttcagacgtttctaacaag

SEQ ID NO: 50 - DNA, 20 bp, synthetic construct
  source 1..20: mol_type = other DNA
ctttgtacagaattctttgg

SEQ ID NO: 51 - DNA, 18 bp, synthetic construct
  source 1..18: mol_type = other DNA
tgctcacctttcctgaac

SEQ ID NO: 52 - DNA, 22 bp, synthetic construct
  source 1..22: mol_type = other DNA
ccactgataaatgggatttgag

SEQ ID NO: 53 - DNA, 20 bp, synthetic construct
  source 1..20: mol_type = other DNA
atagcatttgcagtagctcc